European Patent Specification EP 3 619 303 B1, published June 7, 2023. Title: SESQUITERPENE SYNTHASES FOR PRODUCTION OF DRIMENOL AND MIXTURES THEREOF. Applicant: Firmenich SA Li, Pan Wang, Qi He, Xiu-Feng Haefliger, Olivier. The sequence listing filed with the application follows.

SEQUENCE LISTING (5 sequences)

SEQ ID NO: 1 - DNA, 1674 bp, Paeonia anomala
  misc_feature: cDNA
atgtctgtcaaagttcctcaatctcagaatgctcctacagaggttggacgtcggtccgtaaattttcatcctactgtttggggagatcggtttatcacatacaataaccagtcagttgatgatgatgtggaaaagagattaacaaaagaactaaaatcccaagtgaggagaaagttggtggatgctgctgaaaatacatgtcagaagcttaacacaatcgatgcaatcgagagattaggcttggcttatcatttcgaaacagagattgaagaagcactgcaaaatatttataattcctctcaggttgttggaaataatgtggaagaagatgacctctactctgttgccttacgctttaggcttctcagacaacagggctacaatatttcatctgatgtgtttaacaaattcaaagatgataaagataacttcaaggtatctttaattggtgatgcatcaagcttgctaagcctatatgaagctgcacaccttcgagtacacggagaacacatactggatgaagctctaactttctcagttaataatctggaatcaatggcaacccaattaagtccaccccttgcaacacatgtaacccatgcactaaacagaccacttcgaaagggcattccaaggctagaagcaaggcactacatttctgtctacgaacaagatcctttacacgatgaagatctattgaagctcgcaaagttagatttcaaccaattacagaaaattcaccagaaggagctaagcgagatctcaaagtggtggaaagatataaactttgtatcaaagctaccttttgcaagggacagagtggtggagtgctacttttggataatgtcagtgcatagcgagcccgagaactggcttgcacgaaggacagctgcaaaaatagctgcggtaacctccattatagatgatatctatgatgtgcatggtacaattgacgaactgacgctatttacagaagccgtcaacaggtgggatataaacaacattgatcaactcccggagtacatgaaaatatgttataaggcgctcttgggcgtttttagtgaattaggggaagagttggaaaaacaaggaagatcttaccgcctcgatcatacaattgaacttatgaaagatctagttgggaactattttactgaatcgaaatggttaagcgaaaaatatgtgcccacaatagaggagtatatgcgtgctgcagaagtcaccataggttacaacaatgctataactgcatcttttgccacagccaaagccggagatattgcaaccaaggagacctttgaatgggtgttgagtgaacctaaaattgttaaggcttcctcagtaatttgcaggttgatggatgacttatcatcccacaagtttgagcaaaagagaggacatgttgcatctgctattgaatgctacatgaagcaacatgatgctacagaggaaaaggtgcgtgcggagtttaataaacaagtcaccgacgcctggaaggtgataaatcaagaatgtctccacccaacagccattccaatgcctcttcttacatgtgttctcaactatgcacgtgtggctgatgtcatgtacaaggatggagatgcttatacatttgcccagatcttactgaaagatcatttatcggcattgttcaccgatcctattgcaatgtga

SEQ ID NO: 2 - protein, 557 aa, Paeonia anomala
MSVKVPQSQNAPTEVGRRSVNFHPTVWGDRFITYNNQSVDDDVEKRLTKELKSQVRRKLVDAAENTCQKLNTIDAIERLGLAYHFETEIEEALQNIYNSSQVVGNNVEEDDLYSVALRFRLLRQQGYNISSDVFNKFKDDKDNFKVSLIGDASSLLSLYEAAHLRVHGEHILDEALTFSVNNLESMATQLSPPLATHVTHALNRPLRKGIPRLEARHYISVYEQDPLHDEDLLKLAKLDFNQLQKIHQKELSEISKWWKDINFVSKLPFARDRVVECYFWIMSVHSEPENWLARRTAAKIAAVTSIIDDIYDVHGTIDELTLFTEAVNRWDINNIDQLPEYMKICYKALLGVFSELGEELEKQGRSYRLDHTIELMKDLVGNYFTESKWLSEKYVPTIEEYMRAAEVTIGYNNAITASFATAKAGDIATKETFEWVLSEPKIVKASSVICRLMDDLSSHKFEQKRGHVASAIECYMKQHDATEEKVRAEFNKQVTDAWKVINQECLHPTAIPMPLLTCVLNYARVADVMYKDGDAYTFAQILLKDHLSALFTDPIAM

SEQ ID NO: 3 - DNA, 1674 bp, Artificial Sequence
  codon optimized sequence
atgtccgttaaagttccgcaaagccaaaatgcccctaccgaagttggccgtcgttccgtcaacttccacccgacggtctggggtgatcgtttcattacctacaataaccagagcgttgacgacgatgtggaaaagcgtttgaccaaagaattgaagtcccaggtccgtcgtaaactggttgacgctgcagagaacacttgccagaaactgaacaccatcgacgcgatcgagcgcctgggtctggcttaccatttcgagactgagattgaagaggcactgcagaacatctacaattccagccaagtcgtgggcaataatgtagaggaagatgatttatatagcgtggcgctgcgttttcgtctgctgcgtcaacagggttataacatcagctccgatgtctttaacaagttcaaagatgataaagacaatttcaaggttagcctgatcggtgacgcaagctctttgttatctctgtatgaagccgcgcatctgcgcgtgcatggcgagcatatcttggatgaagcgctgacctttagcgttaataatctggaatcgatggcaacccagctgagcccgccgctggcaacgcacgttacgcacgcgttgaaccgcccgctgcgcaagggtatcccgcgtctggaagcgcgtcattacatttctgtgtacgaacaagatccactgcacgacgaagatttgcttaaactggcgaaactggattttaatcaactgcaaaagattcaccagaaagaactgagcgagattagcaaatggtggaaagacattaatttcgtcagcaagctgccgttcgcccgcgaccgtgttgtggagtgctatttctggattatgagcgttcacagcgagcctgagaactggctggcgcgccgcaccgcggctaagattgcggcagtcacgtcgattatcgacgatatctatgacgtccacggcaccatcgatgaactgacgctgttcaccgaagccgttaaccgctgggacatcaacaacattgatcagctgccggaatacatgaagatctgctacaaagcgctgctgggcgtgttcagcgagctgggtgaagaactggagaaacagggtcgtagctatcgcttggatcataccattgagctgatgaaagatctggtcggtaattacttcaccgagtccaagtggctgagcgagaaatacgttccgacgatcgaagagtacatgcgtgctgccgaagtgaccatcggttacaacaatgccattacggcatcttttgccacggcaaaggccggtgatatcgctaccaaagaaacctttgaatgggtgctgagcgaaccgaagattgtcaaagcctccagcgttatttgtcgtctgatggacgatttgagcagccataagtttgagcaaaagcgtggccacgtcgcgagcgcgatcgagtgctatatgaaacagcacgacgcgaccgaggaaaaagttcgtgcagagttcaataaacaagtcaccgatgcgtggaaagtcattaaccaagagtgcttgcacccgacggcgatcccgatgccactgctgacctgtgtgctcaattatgcacgtgttgcggacgttatgtataaggatggtgacgcgtatacctttgcgcaaattctgctgaaagaccacctgagcgcactgttcacggacccgatcgcgatgtaa

SEQ ID NO: 4 - DNA, 23 bp, Artificial Sequence
  Primer
atgtctgtcaaagttcctcaatc

SEQ ID NO: 5 - DNA, 22 bp, Artificial Sequence
  Primer
tcacattgcaataggatcggtg